European Patent Application EP 4 455 306 A1, published October 30, 2024. Title: 单细胞核酸标记和分析方法. Applicant: 深圳华大生命科学研究院. Application CN. The sequence listing filed with the application follows.

SEQUENCE LISTING (22 sequences)

SEQ ID NO: 1 - DNA, 171 bp, synthetic construct
  source 1..171: mol_type = other DNA; note = library of DNA molecules
gaacgacatggctacgatccgacttnnnnnnnnnnnnnnnnnaagtcggaggccaagcggtcttaggaagacaannnnnnnnnnnnnnnnnnnnnnnnnctgataaggtcgccatgcctctcagtacgtcagcagttnnnnnnnnnnnnnnnnncaactccttggctcaca

SEQ ID NO: 2 - DNA, 24 bp, synthetic construct
  source 1..24: mol_type = other DNA; note = DNB primer
gccatgtcgttcggaaccgagtgt

SEQ ID NO: 3 - DNA, 36 bp, synthetic construct
  source 1..36: mol_type = other DNA; note = Primer for synthesizing chip sequence
ctgctgacgtactgagaggcatggcgaccttatcag

SEQ ID NO: 4 - DNA, 36 bp, synthetic construct; identical to SEQ ID NO: 3
  source 1..36: mol_type = other DNA; note = common sequence X1

SEQ ID NO: 5 - DNA, 13 bp, synthetic construct
  source 1..13: mol_type = other DNA; note = common sequence X2
ttgtcttcctaag

SEQ ID NO: 6 - DNA, 54 bp, synthetic construct
  source 1..54: mol_type = other DNA; note = polyT primer
accgcttggcctccgnnnnnnnnnnttttttttttttttttttttttttttttv

SEQ ID NO: 7 - DNA, 30 bp, synthetic construct
  source 1..30: mol_type = other DNA; note = TSO
aagcagtggtatcaacgcagagtacatggg

SEQ ID NO: 8 - DNA, 76 bp, synthetic construct
  source 1..76: mol_type = other DNA; note = chip sequence
ctgctgacgtactgagaggcatggcgaccttatcagnnnnnnnnnnnnnnnnnnnnnnnnnttgtcttcctaagac

SEQ ID NO: 9 - DNA, 24 bp, synthetic construct
  source 1..24: mol_type = other DNA; note = the bridging oligonucleotide
aggccaagcggtcttaggaagaca

SEQ ID NO: 10 - DNA, 23 bp, synthetic construct
  source 1..23: mol_type = other DNA; note = cDNA amplification primer (1)
ctgctgacgtactgagaggcatg

SEQ ID NO: 11 - DNA, 25 bp, synthetic construct
  source 1..25: mol_type = other DNA; note = cDNA amplification primer (2)
aagcagtggtatcaacgcagagtac

SEQ ID NO: 12 - DNA, 22 bp, synthetic construct
  source 1..22: mol_type = other DNA; note = primer-1 for library construction
ctgctgacgtactgagaggcat

SEQ ID NO: 13 - DNA, 24 bp, synthetic construct
  source 1..24: mol_type = other DNA; note = primer-2 for library construction
gagacgttctcgactcagaagatg

SEQ ID NO: 14 - DNA, 24 bp, synthetic construct
  source 1..24: mol_type = other DNA; note = primer for synthesizing DNB for sequencing
ggcctccgacttgagacgttctcg

SEQ ID NO: 15 - DNA, 48 bp, synthetic construct
  source 1..48: mol_type = other DNA; note = the capture sequence of probe
ttgtcttcctaagacnnnnnnnnnnttttttttttttttttttttttv

SEQ ID NO: 16 - DNA, 109 bp, synthetic construct
  source 1..109: mol_type = other DNA; note = the probe sequence
ctgctgacgtactgagaggcatggcgaccttatcagnnnnnnnnnnnnnnnnnnnnnnnnnttgtcttcctaagacnnnnnnnnnnttttttttttttttttttttttv

SEQ ID NO: 17 - DNA, 23 bp, synthetic construct
  source 1..23: mol_type = other DNA; note = TSO
ctgctgacgtactgagaggcggg

SEQ ID NO: 18 - DNA, 23 bp, synthetic construct
  source 1..23: mol_type = other DNA; note = cDNA amplification primer
ctgctgacgtactgagaggcatg

SEQ ID NO: 19 - DNA, 41 bp, synthetic construct
  source 1..41: mol_type = other DNA; note = the first chain for Tn5 packeting
gagacgttctcgactcagcagaagatgtgtataagagacag

SEQ ID NO: 20 - DNA, 19 bp, synthetic construct
  source 1..19: mol_type = other DNA; note = the second chain for Tn5 packeting
ctgtctcttatacacatct

SEQ ID NO: 21 - DNA, 22 bp, synthetic construct
  source 1..22: mol_type = other DNA; note = primer-2 for library construction
gagacgttctcgactcagcaga

SEQ ID NO: 22 - DNA, 24 bp, synthetic construct
  source 1..24: mol_type = other DNA; note = primer for synthesizing DNB for sequencing
gtacgtcagcaggagacgttctcg